European Patent Specification EP 4 370 145 B1, published August 26, 2026. Title: IMMUNOTHERAPEUTIC METHOD FOR INCREASING CASHEW TOLERANCE IN A SUBJECT. Applicant: DBV TECHNOLOGIES. The sequence listing filed with the application follows.

SEQUENCE LISTING (8 sequences)

SEQ ID NO: 1 - protein, 26 aa, Artificial Sequence
  Human regulatory Treg epitope
PAVLQSSGLYSLSSVVTVPSSSLGTQ

SEQ ID NO: 2 - protein, 21 aa, Artificial Sequence
  Human regulatory Treg epitope
EEQYNSTYRVVSVLTVLHQDW

SEQ ID NO: 3 - protein, 15 aa, Artificial Sequence
  Human regulatory Treg epitope
GTDFTLTISSLQPED

SEQ ID NO: 4 - protein, 20 aa, Artificial Sequence
  murine regulatory Treg epitope
PAVLQSDLYTLSSSVTVPSS

SEQ ID NO: 5 - protein, 19 aa, Artificial Sequence
  murine regulatory Treg epitope
EEQFNSTFRSVSELPIMHQ

SEQ ID NO: 6 - protein, 26 aa, Artificial Sequence
  regulatory Treg epitope
  D-aminoacid (1)..(26)
QTGLSSSPVTVVSSLSYLGSSQLVAP

SEQ ID NO: 7 - protein, 21 aa, Artificial Sequence
  regulatory Treg epitope
  D-aminoacid (1)..(21)
WDQHLVTLVSVVRYTSNYQEE

SEQ ID NO: 8 - protein, 15 aa, Artificial Sequence
  regulatory Treg epitope
  D-aminoacid (1)..(15)
DEPQLSSITLTFDTG